European Patent Specification EP 4 308 715 B1, published May 13, 2026. Title: Molécule hybride comprenant un fragment Fc d'anticorps et au moins un peptide citrulliné dérivé de la fibrine, et ses utilisations. Applicant: ARTHRITIS RECHERCHE & DEVELOPPEMENT UNIVERSITE DE TOULOUSE III INSERM CENTRE HOSPITALER UNIVERSITAIRE DE TOULOUSE CENTRE HOSPITALER UNIVERSITAIRE DE MONTPELLIER UNIVERSITE DE MONTPELLIER. The sequence listing filed with the application follows.

SEQUENCE LISTING (31 sequences)

SEQ ID NO: 1 - protein, 15 aa, Artificial sequence
  Peptide citrulliné
  X (1)..(1): X = résidu citrullyl ou arginyl
  X (13)..(13): X = résidu citrullyl ou arginyl
  X (15)..(15): X = résidu citrullyl ou arginyl
XPAPPPISGGGYXAX

SEQ ID NO: 2 - protein, 15 aa, Artificial sequence
  Peptide citrulliné
  X (3)..(3): X = résidu citrullyl ou arginyl
  X (7)..(7): X = résidu citrullyl ou arginyl
GPXVVEXHQSACKDS

SEQ ID NO: 3 - protein, 15 aa, Artificial sequence
  Peptide citrulliné
  X (10)..(10): X = résidu citrullyl ou arginyl
  X (12)..(12): X = résidu citrullyl ou arginyl
SGIGTLDGFXHXHPD

SEQ ID NO: 4 - protein, 15 aa, Artificial sequence
  Peptide citrulliné
  X (8)..(8): X = résidu citrullyl ou arginyl
  X (11)..(11): X = résidu citrullyl ou arginyl
VDIDIKIXSCXGSCS

SEQ ID NO: 5 - protein, 15 aa, Artificial sequence
  Peptide citrulliné
  X (3)..(3): X = résidu citrullyl
  X (7)..(7): X = résidu citrullyl
GPXVVEXHQSACKDS

SEQ ID NO: 6 - protein, 15 aa, Artificial sequence
  Peptide citrulliné
  X (8)..(8): X = résidu citrullyl
  X (11)..(11): X = résidu citrullyl
VDIDIKIXSCXGSCS

SEQ ID NO: 7 - protein, 15 aa, Artificial sequence
  Peptide citrulliné
  x (4)..(4): X = résidu citrullyl
  x (8)..(8): X = résidu citrullyl
SCSXALAXEVDLKDY

SEQ ID NO: 8 - protein, 15 aa, Artificial sequence
  Peptide citrulliné
  X (13)..(13): X = résidu citrullyl
PEWKALTDMPQMXME

SEQ ID NO: 9 - protein, 15 aa, Artificial sequence
  Peptide citrulliné
  X (5)..(5): X = résidu citrullyl
  X (13)..(13): X = résidu citrullyl
MELEXPGGNEITXGG

SEQ ID NO: 10 - protein, 15 aa, Artificial sequence
  Peptide citrulliné
  X (2)..(2): X = résidu citrullyl
EXGSAGHWTSESSVS

SEQ ID NO: 11 - protein, 15 aa, Artificial sequence
  Peptide citrulliné
  X (9)..(9): X = résidu citrullyl
DSPGSGNAXPNNPDW

SEQ ID NO: 12 - protein, 15 aa, Artificial sequence
  Peptide citrulliné
  X (1)..(1): X = résidu citrullyl ou arginyl
  X (7)..(7): X = résidu citrullyl ou arginyl
  X (10)..(10): X = résidu citrullyl ou arginyl
XGHAKSXPVXGIHTS

SEQ ID NO: 13 - protein, 15 aa, Artificial sequence
  Peptide citrulliné
  X (15)..(15): X = résidu citrullyl
GTFEEVSGNVSPGTX

SEQ ID NO: 14 - protein, 15 aa, Artificial sequence
  Peptide citrulliné
  X (10)..(10): X = résidu citrullyl
  X (12)..(12): X = résidu citrullyl
SGIGTLDGFXHXHPD

SEQ ID NO: 15 - protein, 15 aa, Artificial sequence
  Peptide citrulliné
  X (2)..(2): X = résidu citrullyl
SXGSESGIFTNTKES

SEQ ID NO: 16 - protein, 15 aa, Artificial sequence
  Peptide citrulliné
  X (13)..(13): X = résidu citrullyl
SSHHPGIAEFPSXGK

SEQ ID NO: 17 - protein, 15 aa, Artificial sequence
  Peptide citrulliné
  X (4)..(4): X = résidu citrullyl
SYNXGDSTFESKSYK

SEQ ID NO: 18 - protein, 15 aa, Artificial sequence
  Peptide citrulliné
  X (1)..(1): X = résidu citrullyl
  X (7)..(7): X = résidu citrullyl
  X (10)..(10): X = résidu citrullyl
XGHAKSXPVXGIHTS

SEQ ID NO: 19 - protein, 15 aa, Artificial sequence
  Peptide citrulliné
  X (1)..(1): X = résidu citrullyl
  X (13)..(13): X = résidu citrullyl
  X (15)..(15): X = résidu citrullyl
XPAPPPISGGGYXAX

SEQ ID NO: 20 - protein, 15 aa, Artificial sequence
  Peptide citrulliné
  X = résidu citrullyl (15)..(15): X = résidu citrullyl
QKLESDVSAQMEYCX

SEQ ID NO: 21 - protein, 15 aa, Artificial sequence
  Peptide citrulliné
  X (5)..(5): X = résidu citrullyl
  X (14)..(14): X = résidu citrullyl
VIQNXQDGSVDFGXK

SEQ ID NO: 22 - protein, 15 aa, Artificial sequence
  Peptide citrulliné
  X (2)..(2): X = résidu citrullyl
PXKQCSKEDGGGWWY

SEQ ID NO: 23 - protein, 15 aa, Artificial sequence
  Peptide citrulliné
  X (4)..(4): X = résidu citrullyl
  X (13)..(13): X = résidu citrullyl
WYNXCHAANPNGXYY

SEQ ID NO: 24 - protein, 217 aa, Homo sapiens
APELLGGPSVFLFPPKPKDTLMISRTPEVTCVVVDVSHEDPEVKFNWYVDGVEVHNAKTKPREEQYNSTYRVVSVLTVLHQDWLNGKEYKCKVSNKALPAPIEKTISKAKGQPREPQVYTLPPSREEMTKNQVSLTCLVKGFYPSDIAVEWESNGQPENNYKTTPPVLDSDGSFFLYSKLTVDKSRWQQGNVFSCSVMHEALHNHYTQKSLSLSPGK

SEQ ID NO: 25 - protein, 234 aa, Artificial sequence
  Fragment Fc + Qtag
LLQGARSDATHTCPPCPAPELLGGPSVFLFPPKPKDTLMISRTPEVTCVVVDVSHEDPEVKFNWYVDGVEVHNAKTKPREEQYNSTYRVVSVLTVLHQDWLNGKEYKCKVSNKALPAPIEKTISKAKGQPREPQVYTLPPSREEMTKNQVSLTCLVKGFYPSDIAVEWESNGQPENNYKTTPPVLDSDGSFFLYSKLTVDKSRWQQGNVFSCSVMHEALHNHYTQKSLSLSPGK

SEQ ID NO: 26 - protein, 241 aa, Artificial sequence
  Fragment Fc + Qtag
AHGHGHGLLQGARSDATHTCPPCPAPELLGGPSVFLFPPKPKDTLMISRTPEVTCVVVDVSHEDPEVKFNWYVDGVEVHNAKTKPREEQYNSTYRVVSVLTVLHQDWLNGKEYKCKVSNKALPAPIEKTISKAKGQPREPQVYTLPPSREEMTKNQVSLTCLVKGFYPSDIAVEWESNGQPENNYKTTPPVLDSDGSFFLYSKLTVDKSRWQQGNVFSCSVMHEALHNHYTQKSLSLSPGK

SEQ ID NO: 27 - protein, 600 aa, Homo sapiens
GPRVVERHQSACKDSDWPFCSDEDWNYKCPSGCRMKGLIDEVNQDFTNRINKLKNSLFEYQKNNKDSHSLTTNIMEILRGDFSSANNRDNTYNRVSEDLRSRIEVLKRKVIEKVQHIQLLQKNVRAQLVDMKRLEVDIDIKIRSCRGSCSRALAREVDLKDYEDQQKQLEQVIAKDLLPSRDRQHLPLIKMKPVPDLVPGNFKSQLQKVPPEWKALTDMPQMRMELERPGGNEITRGGSTSYGTGSETESPRNPSSAGSWNSGSSGPGSTGNRNPGSSGTGGTATWKPGSSGPGSTGSWNSGSSGTGSTGNQNPGSPRPGSTGTWNPGSSERGSAGHWTSESSVSGSTGQWHSESGSFRPDSPGSGNARPNNPDWGTFEEVSGNVSPGTRREYHTEKLVTSKGDKELRTGKEKVTSGSTTTTRRSCSKTVTKTVIGPDGHKEVTKEVVTSEDGSDCPEAMDLGTLSGIGTLDGFRHRHPDEAAFFDTASTGKTFPGFFSPMLGEFVSETESRGSESGIFTNTKESSSHHPGIAEFPSRGKSSSYSKQFTSSTSYNRGDSTFESKSYKMADEAGSEADHEGTHSTKRGHAKSRPVRGIHTS

SEQ ID NO: 28 - protein, 447 aa, Homo sapiens
GHRPLDKKREEAPSLRPAPPPISGGGYRARPAKAAATQKKVERKAPDAGGCLHADPDLGVLCPTGCQLQEALLQQERPIRNSVDELNNNVEAVSQTSSSSFQYMYLLKDLWQKRQKQVKDNENVVNEYSSELEKHQLYIDETVNSNIPTNLRVLRSILENLRSKIQKLESDVSAQMEYCRTPCTVSCNIPVVSGKECEEIIRKGGETSEMYLIQPDSSVKPYRVYCDMNTENGGWTVIQNRQDGSVDFGRKWDPYKQGFGNVATNTDGKNYCGLPGEYWLGNDKISQLTRMGPTELLIEMEDWKGDKVKAHYGGFTVQNEANKYQISVNKYRGTAGNALMDGASQLMGENRTMTIHNGMFFSTYDRDNDGWLTSDPRKQCSKEDGGGWWYNRCHAANPNGRYYWGGQYTWDMAKHGTDDGVVWMNWKGSWYSMRKMSMKIRPFFPQQ

SEQ ID NO: 29 - protein, 4 aa, Artificial sequence
  Qtag
LLQG

SEQ ID NO: 30 - protein, 635 aa, Homo sapiens
MFSMRIVCLVLSVVGTAWTADSGEGDFLAEGGGVRGPRVVERHQSACKDSDWPFCSDEDWNYKCPSGCRMKGLIDEVNQDFTNRINKLKNSLFEYQKNNKDSHSLTTNIMEILRGDFSSANNRDNTYNRVSEDLRSRIEVLKRKVIEKVQHIQLLQKNVRAQLVDMKRLEVDIDIKIRSCRGSCSRALAREVDLKDYEDQQKQLEQVIAKDLLPSRDRQHLPLIKMKPVPDLVPGNFKSQLQKVPPEWKALTDMPQMRMELERPGGNEITRGGSTSYGTGSETESPRNPSSAGSWNSGSSGPGSTGNRNPGSSGTGGTATWKPGSSGPGSTGSWNSGSSGTGSTGNQNPGSPRPGSTGTWNPGSSERGSAGHWTSESSVSGSTGQWHSESGSFRPDSPGSGNARPNNPDWGTFEEVSGNVSPGTRREYHTEKLVTSKGDKELRTGKEKVTSGSTTTTRRSCSKTVTKTVIGPDGHKEVTKEVVTSEDGSDCPEAMDLGTLSGIGTLDGFRHRHPDEAAFFDTASTGKTFPGFFSPMLGEFVSETESRGSESGIFTNTKESSSHHPGIAEFPSRGKSSSYSKQFTSSTSYNRGDSTFESKSYKMADEAGSEADHEGTHSTKRGHAKSRPVRGIHTS

SEQ ID NO: 31 - protein, 491 aa, Homo sapiens
MKRMVSWSFHKLKTMKHLLLLLLCVFLVKSQGVNDNEEGFFSARGHRPLDKKREEAPSLRPAPPPISGGGYRARPAKAAATQKKVERKAPDAGGCLHADPDLGVLCPTGCQLQEALLQQERPIRNSVDELNNNVEAVSQTSSSSFQYMYLLKDLWQKRQKQVKDNENVVNEYSSELEKHQLYIDETVNSNIPTNLRVLRSILENLRSKIQKLESDVSAQMEYCRTPCTVSCNIPVVSGKECEEIIRKGGETSEMYLIQPDSSVKPYRVYCDMNTENGGWTVIQNRQDGSVDFGRKWDPYKQGFGNVATNTDGKNYCGLPGEYWLGNDKISQLTRMGPTELLIEMEDWKGDKVKAHYGGFTVQNEANKYQISVNKYRGTAGNALMDGASQLMGENRTMTIHNGMFFSTYDRDNDGWLTSDPRKQCSKEDGGGWWYNRCHAANPNGRYYWGGQYTWDMAKHGTDDGVVWMNWKGSWYSMRKMSMKIRPFFPQQ